European Patent Application EP 4 324 922 A1, published February 21, 2024. Title: METHOD AND DEVICE OF PROCESSING INFORMATION. Applicant: KYOTO UNIVERSITY. The sequence listing filed with the application follows.

SEQUENCE LISTING (3 sequences)

SEQ ID NO: 1 - DNA, 23 bp, Artificial Sequence
  Synthesized nucleotides
tccaaggagctgcaggcggcgca

SEQ ID NO: 2 - DNA, 28 bp, Artificial Sequence
  Synthesized nucleotides
acagaattcgccccggcctggtacactg

SEQ ID NO: 3 - DNA, 29 bp, Homo sapiens
atctcagaaaaaaaaaaaattctctatct